European Patent Application EP 4 253 537 A1, published October 4, 2023. Title: Method, Device, Program and Recording Medium for Designing Amplicon Methylation Sequence Analytical Primer and Method for Manufacturing Amplicon Methylation Sequence Analytical Primer. Applicant: Fuji Film Corporation. The sequence listing filed with the application follows.

SEQUENCE LISTING (148 sequences)

SEQ ID NO: 1 - DNA, 22 bp, Artificial Sequence
  Human Chr.16
ttatttttgggaatagtttgga

SEQ ID NO: 2 - DNA, 27 bp, Artificial Sequence
  Human Chr.3
ttttaattattattttattttgaagga

SEQ ID NO: 3 - DNA, 25 bp, Artificial Sequence
  Human Chr.3
gagtatattttttttggtttaaaga

SEQ ID NO: 4 - DNA, 26 bp, Artificial Sequence
  Human Chr.1
ggaaataaagttaagtgtagttagga

SEQ ID NO: 5 - DNA, 30 bp, Artificial Sequence
  Human Chr.8
tttttaaaataaattatattaaggtaagaa

SEQ ID NO: 6 - DNA, 22 bp, Artificial Sequence
  Human Chr.14
gataaatggaaaaaaagaggaa

SEQ ID NO: 7 - DNA, 21 bp, Artificial Sequence
  Human Chr.16
tagagttttgtggagggaaga

SEQ ID NO: 8 - DNA, 23 bp, Artificial Sequence
  Human Chr.8
ttttaattaataggggtttagga

SEQ ID NO: 9 - DNA, 23 bp, Artificial Sequence
  Human Chr.1
tgtggttatagtggtaagtagga

SEQ ID NO: 10 - DNA, 24 bp, Artificial Sequence
  Human Chr.6
gataagataggagttttgtgaaga

SEQ ID NO: 11 - DNA, 28 bp, Artificial Sequence
  Human Chr.2
tagttttatttttttattttgtagaaga

SEQ ID NO: 12 - DNA, 23 bp, Artificial Sequence
  Human Chr.4
ttggttagatgtttgtagtagga

SEQ ID NO: 13 - DNA, 28 bp, Artificial Sequence
  Human Chr.11
atttagtttattttgaattattatgaga

SEQ ID NO: 14 - DNA, 20 bp, Artificial Sequence
  Human Chr.1
aattatgtgggaggtaggga

SEQ ID NO: 15 - DNA, 20 bp, Artificial Sequence
  Human Chr.8
tagtggaaaagaatgggaga

SEQ ID NO: 16 - DNA, 22 bp, Artificial Sequence
  Human Chr.14
taaatgggttagttttgaaaga

SEQ ID NO: 17 - DNA, 21 bp, Artificial Sequence
  Human Chr.20
taggtagggtggaaaaaagaa

SEQ ID NO: 18 - DNA, 29 bp, Artificial Sequence
  Human Chr.1
gaggatatatgtagtaattttttaagaga

SEQ ID NO: 19 - DNA, 23 bp, Artificial Sequence
  Human Chr.1
ttagtaagggggattttattaga

SEQ ID NO: 20 - DNA, 23 bp, Artificial Sequence
  Human Chr.1
tggtaataaaatggtgaataaga

SEQ ID NO: 21 - DNA, 25 bp, Artificial Sequence
  Human Chr.10
aatgtttatagatagtgaaaaggaa

SEQ ID NO: 22 - DNA, 29 bp, Artificial Sequence
  Human Chr.1
agtgaagatagtataagtaaaagatagga

SEQ ID NO: 23 - DNA, 22 bp, Artificial Sequence
  Human Chr.2
aattgggtatttaaatgggaga

SEQ ID NO: 24 - DNA, 27 bp, Artificial Sequence
  Human Chr.12
tttttgtttttatttttaatagtagga

SEQ ID NO: 25 - DNA, 24 bp, Artificial Sequence
  Human Chr.16
tttttataattaggttaaagggaa

SEQ ID NO: 26 - DNA, 25 bp, Artificial Sequence
  Human Chr.10
ttttgagggaaaataattttaagaa

SEQ ID NO: 27 - DNA, 30 bp, Artificial Sequence
  Human Chr.18
tgatttaattaaagtttatagtaattttga

SEQ ID NO: 28 - DNA, 22 bp, Artificial Sequence
  Human Chr.21
atttaaaggttttgaggaagga

SEQ ID NO: 29 - DNA, 24 bp, Artificial Sequence
  Human Chr.2
tttggagttatagttagttaggga

SEQ ID NO: 30 - DNA, 22 bp, Artificial Sequence
  Human Chr.8
tgatggaaatttaggtagaaga

SEQ ID NO: 31 - DNA, 24 bp, Artificial Sequence
  Human Chr.3
ttgattgtaaagtgttattaagga

SEQ ID NO: 32 - DNA, 30 bp, Artificial Sequence
  Human Chr.10
ttagttagaattttatttaagtttaagaga

SEQ ID NO: 33 - DNA, 22 bp, Artificial Sequence
  Human Chr.2
ttttggtttttaggagtgaaga

SEQ ID NO: 34 - DNA, 25 bp, Artificial Sequence
  Human Chr.7
ggaataatgtttaggtagtttagga

SEQ ID NO: 35 - DNA, 21 bp, Artificial Sequence
  Human Chr.3
agggattagagtgagaaggaa

SEQ ID NO: 36 - DNA, 22 bp, Artificial Sequence
  Human Chr.16
tggaagagttataatttaggga

SEQ ID NO: 37 - DNA, 22 bp, Artificial Sequence
  Human Chr.1
ttagggatttttatggtagaga

SEQ ID NO: 38 - DNA, 24 bp, Artificial Sequence
  Human Chr.1
agttttttatattgaggtaaagga

SEQ ID NO: 39 - DNA, 26 bp, Artificial Sequence
  Human Chr.17
ggtatggaatgtgtttatagataaga

SEQ ID NO: 40 - DNA, 20 bp, Artificial Sequence
  Human Chr.16
taactcccctaatttcacca

SEQ ID NO: 41 - DNA, 20 bp, Artificial Sequence
  Human Chr.3
cctactcacctattacccca

SEQ ID NO: 42 - DNA, 23 bp, Artificial Sequence
  Human Chr.3
aaatattctccaactctatccac

SEQ ID NO: 43 - DNA, 23 bp, Artificial Sequence
  Human Chr.1
ttctatttcatttcaaaaaaaca

SEQ ID NO: 44 - DNA, 21 bp, Artificial Sequence
  Human Chr.8
tctaacccaccaatttataca

SEQ ID NO: 45 - DNA, 23 bp, Artificial Sequence
  Human Chr.14
aactaacaaacacacatacacca

SEQ ID NO: 46 - DNA, 22 bp, Artificial Sequence
  Human Chr.16
ctcttccaaaaaacacttacca

SEQ ID NO: 47 - DNA, 21 bp, Artificial Sequence
  Human Chr.8
taccccaatattaaaaaccac

SEQ ID NO: 48 - DNA, 21 bp, Artificial Sequence
  Human Chr.1
ttcactaacaacccaaaaaca

SEQ ID NO: 49 - DNA, 28 bp, Artificial Sequence
  Human Chr.6
cacactaaataaaacatataatttaaca

SEQ ID NO: 50 - DNA, 24 bp, Artificial Sequence
  Human Chr.2
aaataacctctataatccactcac

SEQ ID NO: 51 - DNA, 21 bp, Artificial Sequence
  Human CHr.4
aactaaccccaaatttaacca

SEQ ID NO: 52 - DNA, 22 bp, Artificial Sequence
  Human Chr.11
tcccatctacaccttataaaca

SEQ ID NO: 53 - DNA, 25 bp, Artificial Sequence
  Human Chr.1
aactaactaccatactactaaccca

SEQ ID NO: 54 - DNA, 24 bp, Artificial Sequence
  Human Chr.8
ttcaacttaactcaattttaaaca

SEQ ID NO: 55 - DNA, 22 bp, Artificial Sequence
  Human Chr.14
acaatttaatttaaaaacccca

SEQ ID NO: 56 - DNA, 22 bp, Artificial Sequence
  Human Chr.20
aatacaaaataatctaacccca

SEQ ID NO: 57 - DNA, 20 bp, Artificial Sequence
  Human Chr.1
ttcattaccccttaatacca

SEQ ID NO: 58 - DNA, 27 bp, Artificial Sequence
  Human Chr.1
aaacttataccaaaaaataataaaaca

SEQ ID NO: 59 - DNA, 27 bp, Artificial Sequence
  Human Chr.1
atactaataaaaaaaaataaaaaccca

SEQ ID NO: 60 - DNA, 29 bp, Artificial Sequence
  Human Chr.10
aaaataaaataaccaatataatctaacac

SEQ ID NO: 61 - DNA, 27 bp, Artificial Sequence
  Human Chr.1
aaaaaactaaactaaactaaacaaaca

SEQ ID NO: 62 - DNA, 24 bp, Artificial Sequence
  Human Chr.2
accaaaaataaatctaaacaaaca

SEQ ID NO: 63 - DNA, 21 bp, Artificial Sequence
  Human Chr.12
cctctctaacctaaaacccac

SEQ ID NO: 64 - DNA, 23 bp, Artificial Sequence
  Human Chr.16
atataaaacaaatctaaccacca

SEQ ID NO: 65 - DNA, 24 bp, Artificial Sequence
  Human Chr.10
cttcatacttacacacacaataca

SEQ ID NO: 66 - DNA, 20 bp, Artificial Sequence
  Human Chr.18
atcaccattaaccaaacaca

SEQ ID NO: 67 - DNA, 21 bp, Artificial Sequence
  Human Chr.21
ataatcctatcaaaaccacca

SEQ ID NO: 68 - DNA, 22 bp, Artificial Sequence
  Human Chr.2
caaacaactaaacataaaccca

SEQ ID NO: 69 - DNA, 21 bp, Artificial Sequence
  Human Chr.8
atctctaaatttttccaacca

SEQ ID NO: 70 - DNA, 20 bp, Artificial Sequence
  Human Chr.3
ctctattttccattcaacca

SEQ ID NO: 71 - DNA, 22 bp, Artificial Sequence
  Human Chr.10
ccaaacataaatcccctataca

SEQ ID NO: 72 - DNA, 20 bp, Artificial Sequence
  Human Chr.2
aaacaataaaccttcccaca

SEQ ID NO: 73 - DNA, 20 bp, Artificial Sequence
  Human Chr.7
catcctacccaacataacca

SEQ ID NO: 74 - DNA, 20 bp, Artificial Sequence
  Human Chr.3
tatactctacctccccaaca

SEQ ID NO: 75 - DNA, 20 bp, Artificial Sequence
  Human Chr.16
accctctcccctaatacaca

SEQ ID NO: 76 - DNA, 22 bp, Artificial Sequence
  Human Chr.1
caaatcattaacttcaaaccac

SEQ ID NO: 77 - DNA, 20 bp, Artificial Sequence
  Human Chr.1
aaaaatttcacaaccaacac

SEQ ID NO: 78 - DNA, 24 bp, Artificial Sequence
  Human Chr.17
caaattccaactcttataaaaaca

SEQ ID NO: 79 - DNA, 22 bp, Artificial Sequence
  Human Chr.16
ttatttttgggaatagtttgga

SEQ ID NO: 80 - DNA, 27 bp, Artificial Sequence
  Human Chr.3
ttttaattattattttattttgaagga

SEQ ID NO: 81 - DNA, 25 bp, Artificial Sequence
  Human Chr.3
gagtatattttttttggtttaaaga

SEQ ID NO: 82 - DNA, 26 bp, Artificial Sequence
  Human Chr.1
ggaaataaagttaagtgtagttagga

SEQ ID NO: 83 - DNA, 30 bp, Artificial Sequence; identical to SEQ ID NO: 5
  Human Chr.8

SEQ ID NO: 84 - DNA, 22 bp, Artificial Sequence
  Human Chr.14
gataaatggaaaaaaagaggaa

SEQ ID NO: 85 - DNA, 21 bp, Artificial Sequence
  Human Chr.16
gggggtaggagagtaaaaaga

SEQ ID NO: 86 - DNA, 23 bp, Artificial Sequence
  Human Chr.2
ttttaattaataggggtttagga

SEQ ID NO: 87 - DNA, 24 bp, Artificial Sequence
  Human Chr.6
gataagataggagttttgtgaaga

SEQ ID NO: 88 - DNA, 28 bp, Artificial Sequence
  Human Chr.2
tagttttatttttttattttgtagaaga

SEQ ID NO: 89 - DNA, 23 bp, Artificial Sequence
  Human Chr.4
ttggttagatgtttgtagtagga

SEQ ID NO: 90 - DNA, 28 bp, Artificial Sequence
  Human Chr.11
atttagtttattttgaattattatgaga

SEQ ID NO: 91 - DNA, 20 bp, Artificial Sequence
  Human Chr.1
aattatgtgggaggtaggga

SEQ ID NO: 92 - DNA, 20 bp, Artificial Sequence
  Human Chr.8
tagtggaaaagaatgggaga

SEQ ID NO: 93 - DNA, 22 bp, Artificial Sequence
  Human Chr.14
taaatgggttagttttgaaaga

SEQ ID NO: 94 - DNA, 29 bp, Artificial Sequence
  Human Chr.1
gaggatatatgtagtaattttttaagaga

SEQ ID NO: 95 - DNA, 23 bp, Artificial Sequence
  Human Chr.1
ttagtaagggggattttattaga

SEQ ID NO: 96 - DNA, 23 bp, Artificial Sequence
  Human Chr.1
tggtaataaaatggtgaataaga

SEQ ID NO: 97 - DNA, 25 bp, Artificial Sequence
  Human Chr.10
aatgtttatagatagtgaaaaggaa

SEQ ID NO: 98 - DNA, 29 bp, Artificial Sequence
  Human Chr.1
agtgaagatagtataagtaaaagatagga

SEQ ID NO: 99 - DNA, 22 bp, Artificial Sequence
  Human Chr.2
aattgggtatttaaatgggaga

SEQ ID NO: 100 - DNA, 24 bp, Artificial Sequence
  Human Chr.16
tttttataattaggttaaagggaa

SEQ ID NO: 101 - DNA, 25 bp, Artificial Sequence
  Human Chr.10
ttttgagggaaaataattttaagaa

SEQ ID NO: 102 - DNA, 30 bp, Artificial Sequence; identical to SEQ ID NO: 27
  Human Chr.18

SEQ ID NO: 103 - DNA, 21 bp, Artificial Sequence
  Human Chr.21
ttatggagaaaagtgaaagga

SEQ ID NO: 104 - DNA, 24 bp, Artificial Sequence
  Human Chr.2
tttggagttatagttagttaggga

SEQ ID NO: 105 - DNA, 26 bp, Artificial Sequence
  Human Chr.8
aaagtttggttattatttttgtaaga

SEQ ID NO: 106 - DNA, 24 bp, Artificial Sequence
  Human Chr.3
ttgattgtaaagtgttattaagga

SEQ ID NO: 107 - DNA, 30 bp, Artificial Sequence; identical to SEQ ID NO: 32
  Human Chr.10

SEQ ID NO: 108 - DNA, 22 bp, Artificial Sequence
  Human Chr.2
ttttggtttttaggagtgaaga

SEQ ID NO: 109 - DNA, 25 bp, Artificial Sequence
  Human Chr.7
ggaataatgtttaggtagtttagga

SEQ ID NO: 110 - DNA, 21 bp, Artificial Sequence
  Human Chr.3
agggattagagtgagaaggaa

SEQ ID NO: 111 - DNA, 22 bp, Artificial Sequence
  Human Chr.16
tggaagagttataatttaggga

SEQ ID NO: 112 - DNA, 22 bp, Artificial Sequence
  Human Chr.1
ttagggatttttatggtagaga

SEQ ID NO: 113 - DNA, 24 bp, Artificial Sequence
  Human Chr.1
agttttttatattgaggtaaagga

SEQ ID NO: 114 - DNA, 20 bp, Artificial Sequence
  Human Chr.16
taactcccctaatttcacca

SEQ ID NO: 115 - DNA, 20 bp, Artificial Sequence
  Human Chr.3
cctactcacctattacccca

SEQ ID NO: 116 - DNA, 23 bp, Artificial Sequence
  Human Chr.3
aaatattctccaactctatccac

SEQ ID NO: 117 - DNA, 24 bp, Artificial Sequence
  Human Chr.1
tttctatttcatttcaaaaaaaca

SEQ ID NO: 118 - DNA, 21 bp, Artificial Sequence
  Human Chr.8
tctaacccaccaatttataca

SEQ ID NO: 119 - DNA, 23 bp, Artificial Sequence
  Human Chr.14
aactaacaaacacacatacacca

SEQ ID NO: 120 - DNA, 28 bp, Artificial Sequence
  Human Chr.16
taaaaatacaaaaaaacattaattacca

SEQ ID NO: 121 - DNA, 22 bp, Artificial Sequence
  Human Chr.8
actaccccaatattaaaaacca

SEQ ID NO: 122 - DNA, 28 bp, Artificial Sequence
  Human Chr.6
cacactaaataaaacatataatttaaca

SEQ ID NO: 123 - DNA, 26 bp, Artificial Sequence
  Human Chr.2
actaaaaaataacctctataatccac

SEQ ID NO: 124 - DNA, 27 bp, Artificial Sequence
  Human Chr.4
aacactataacatatttataacaacca

SEQ ID NO: 125 - DNA, 22 bp, Artificial Sequence
  Human Chr.11
tcccatctacaccttataaaca

SEQ ID NO: 126 - DNA, 25 bp, Artificial Sequence
  Human Chr.1
aactaactaccatactactaaccca

SEQ ID NO: 127 - DNA, 24 bp, Artificial Sequence
  Human Chr.8
ttcaacttaactcaattttaaaca

SEQ ID NO: 128 - DNA, 23 bp, Artificial Sequence
  Human Chr.14
tacaatttaatttaaaaacccca

SEQ ID NO: 129 - DNA, 20 bp, Artificial Sequence
  Human Chr.1
cattaccccttaataccaca

SEQ ID NO: 130 - DNA, 27 bp, Artificial Sequence
  Human Chr.1
aaacttataccaaaaaataataaaaca

SEQ ID NO: 131 - DNA, 28 bp, Artificial Sequence
  Human Chr.1
aatactaataaaaaaaaataaaaaccca

SEQ ID NO: 132 - DNA, 29 bp, Artificial Sequence
  Human Chr.10
aaaataaaataaccaatataatctaacac

SEQ ID NO: 133 - DNA, 28 bp, Artificial Sequence
  Human Chr.1
ataaataaataaatcaaactaataacca

SEQ ID NO: 134 - DNA, 25 bp, Artificial Sequence
  Human Chr.2
taccaaaaataaatctaaacaaaca

SEQ ID NO: 135 - DNA, 23 bp, Artificial Sequence
  Human Chr.16
accaccaaataacttaatttaca

SEQ ID NO: 136 - DNA, 24 bp, Artificial Sequence
  Human Chr.10
cttcatacttacacacacaataca

SEQ ID NO: 137 - DNA, 22 bp, Artificial Sequence
  Human Chr.18
aataatcaccattaaccaaaca

SEQ ID NO: 138 - DNA, 21 bp, Artificial Sequence
  Human Chr.21
taaaactcaccaacttaacca

SEQ ID NO: 139 - DNA, 24 bp, Artificial Sequence
  Human Chr.2
atcaaacaactaaacataaaccca

SEQ ID NO: 140 - DNA, 21 bp, Artificial Sequence
  Human Chr.8
cttaaactccttcaaatccac

SEQ ID NO: 141 - DNA, 20 bp, Artificial Sequence
  Human Chr.3
ctctattttccattcaacca

SEQ ID NO: 142 - DNA, 22 bp, Artificial Sequence
  Human Chr.10
ccaaacataaatcccctataca

SEQ ID NO: 143 - DNA, 29 bp, Artificial Sequence
  Human Chr.2
aattaaataaataaataaaaaatacccca

SEQ ID NO: 144 - DNA, 20 bp, Artificial Sequence
  Human Chr.7
catcctacccaacataacca

SEQ ID NO: 145 - DNA, 20 bp, Artificial Sequence
  Human Chr.3
tatactctacctccccaaca

SEQ ID NO: 146 - DNA, 21 bp, Artificial Sequence
  Human Chr.16
ctcctaaaacaacctacccac

SEQ ID NO: 147 - DNA, 22 bp, Artificial Sequence
  Human Chr.1
caaatcattaacttcaaaccac

SEQ ID NO: 148 - DNA, 20 bp, Artificial Sequence
  Human Chr.1
aaaatttcacaaccaacaca